European Patent Specification EP 2 825 024 B1, published July 12, 2023. Title: Tomato plants with intense phenotype and TYLCV resistance. Applicant: Nunhems B.V. The sequence listing filed with the application follows.

SEQUENCE LISTING (14 sequences)

SEQ ID NO: 1 - DNA, 23 bp, artificial
  Forward primer M-H302A23
tcccgtctcctgcacctacttct

SEQ ID NO: 2 - DNA, 20 bp, artificial
  reverse primer M-H302A23
aaaggggtggtgctcgccct

SEQ ID NO: 3 - DNA, 24 bp, artificial
  forward primer T0774
ctcctcaactggctaattctcagg

SEQ ID NO: 4 - DNA, 25 bp, artificial
  reverse primer T0774
gcaaaccaaatacatcgcgtatcac

SEQ ID NO: 5 - DNA, 25 bp, artificial
  forward primer M-M082G10
ggcatcgccatcatctctaagtcca

SEQ ID NO: 6 - DNA, 24 bp, artificial
  reverse primer M-M082G10
gcctcaacctactgccttgcaaat

SEQ ID NO: 7 - DNA, 21 bp, artificial
  forward primer MSc05732-3
atgcttttcgagcacgagcct

SEQ ID NO: 8 - DNA, 25 bp, artificial
  reverse primer MSc05732-3
agcctaaagagaactaggcagggga

SEQ ID NO: 9 - DNA, 24 bp, artificial
  forward primer MSc05732-4
acgagatggagcggtcttcaagct

SEQ ID NO: 10 - DNA, 24 bp, artificial
  reverse primer MSc05732-4
gacagatctcccggtaggagagca

SEQ ID NO: 11 - DNA, 24 bp, artificial
  forward primer cLEG-31-P16
atggtgactaaggtggatgagcct

SEQ ID NO: 12 - DNA, 24 bp, artificial
  reverse primer cLEG-31-P16
tgagtgccaaccgataatgctacc

SEQ ID NO: 13 - DNA, 21 bp, artificial
  forward primer MSc05732-14
gtggggcctcgatcccagtca

SEQ ID NO: 14 - DNA, 24 bp, artificial
  reverse primer Msc05732-14
ggccctttagtgtgtttcacacct